European Patent Specification EP 2 893 351 B1, published December 6, 2023. Title: Method for identifying subgroups of circulating tumor cells (CTCs) in the CTC population of a biological sample. Applicant: Andreas-Claudius, Hoffmann Jörg Friedrich, Schlaak. The sequence listing filed with the application follows.

SEQUENCE LISTING (2 sequences)

SEQ ID NO: 1 - DNA, 17 bp, Artificial sequence
  Artificial sequence
gagcgcggctacagctt

SEQ ID NO: 2 - DNA, 22 bp, TCCTTAATGTCACGCACGATTT
tccttaatgtcacgcacgattt